European Patent Application EP 4 413 991 A1, published August 14, 2024. Title: Peptide for cognitive improvement. Applicant: CONSEJO SUPERIOR DE INVESTIGACIONES CIENTIFICAS (CSIC). The sequence listing filed with the application follows.

SEQUENCE LISTING (1 sequence)

SEQ ID NO: 1 - protein, 9 aa, synthetic construct
  source 1..9: organism (original language) = constructo sintetico
CTVRTSAEC